European Patent Application EP 4 534 690 A2, published April 9, 2025. Title: SYSTEMS AND METHODS FOR TARGETED NUCLEIC ACID CAPTURE. Applicant: Agilent Technologies, Inc. Application EP. The sequence listing filed with the application follows.

SEQUENCE LISTING (25 sequences)

SEQ ID NO: 1 - DNA, 50 bp, synthetic construct
  misc_feature 1..50: note = Description of Artificial Sequence: Syntheticprobe
  source 1..50: mol_type = other DNA
tttttttttttggcaccagacttaatctaagcagagaacatgataagaga

SEQ ID NO: 2 - DNA, 60 bp, synthetic construct
  misc_feature 1..60: note = Description of Artificial Sequence: Syntheticprobe
  source 1..60: mol_type = other DNA
ctacaacgaagagaattaaggaacttttttttttttttttaccgtggtctgaattagatt

SEQ ID NO: 3 - DNA, 60 bp, synthetic construct
  misc_feature 1..60: note = Description of Artificial Sequence: Syntheticprobe
  source 1..60: mol_type = other DNA
tagctcctaaaggaacaaccgaaagtttttttttttttttcgtctcttgtactattctct

SEQ ID NO: 4 - DNA, 24 bp, synthetic construct
  misc_feature 1..24: note = Description of Artificial Sequence: Syntheticprimer
  source 1..24: mol_type = other DNA
cccgtcgctatcaaggaattaaga

SEQ ID NO: 5 - DNA, 25 bp, synthetic construct
  misc_feature 1..25: note = Description of Artificial Sequence: Syntheticprimer
  source 1..25: mol_type = other DNA
ccacacagcasaagcagaaactcac

SEQ ID NO: 6 - DNA, 120 bp, synthetic construct
  misc_feature 1..120: note = Description of Artificial Sequence: Syntheticprobe
  source 1..120: mol_type = other DNA
agaaggtgagaaagttaaaattcccgtcgctatcaaggaattaagagaagcaacatctccgaaagccaacaaggaaatcctcgatgtgagtttctgctttgctgtgtgggggtccatggc

SEQ ID NO: 7 - DNA, 35 bp, synthetic construct
  misc_feature 1..35: note = Description of Artificial Sequence: Syntheticprobe
  source 1..35: mol_type = other DNA
ttttttttttggtgagaaagttaaaattcccgtcg

SEQ ID NO: 8 - DNA, 35 bp, synthetic construct
  misc_feature 1..35: note = Description of Artificial Sequence: Syntheticprobe
  source 1..35: mol_type = other DNA
tttttttttttcaaggaattaagagaagcaacatc

SEQ ID NO: 9 - DNA, 35 bp, synthetic construct
  misc_feature 1..35: note = Description of Artificial Sequence: Syntheticprobe
  source 1..35: mol_type = other DNA
ttttttttttgaaagccaacaaggaaatcctcgat

SEQ ID NO: 10 - DNA, 35 bp, synthetic construct
  misc_feature 1..35: note = Description of Artificial Sequence: Syntheticprobe
  source 1..35: mol_type = other DNA
ttttttttttagtttctgctttgctgtgtgggggt

SEQ ID NO: 11 - DNA, 94 bp, synthetic construct
  misc_feature 1..94: note = Description of Artificial Sequence: Syntheticprobe
  source 1..94: mol_type = other DNA
ttttttggcaccagacttaatctaatttgcagagaacatgataagagattttggcaccagacttaatctaatttgcagagaacatgataagaga

SEQ ID NO: 12 - DNA, 60 bp, synthetic construct
  misc_feature 1..60: note = Description of Artificial Sequence: Syntheticprobe
  source 1..60: mol_type = other DNA
tctcttatcatgttctctgctttttttttttttttggtgagaaagttaaaattcccgtcg

SEQ ID NO: 13 - DNA, 60 bp, synthetic construct
  misc_feature 1..60: note = Description of Artificial Sequence: Syntheticprobe
  source 1..60: mol_type = other DNA
ttagattaagtctggtgccattttttttttttttttcaaggaattaagagaagcaacatc

SEQ ID NO: 14 - DNA, 60 bp, synthetic construct
  misc_feature 1..60: note = Description of Artificial Sequence: Syntheticprobe
  source 1..60: mol_type = other DNA
tctcttatcatgttctctgctttttttttttttttgaaagccaacaaggaaatcctcgat

SEQ ID NO: 15 - DNA, 60 bp, synthetic construct
  misc_feature 1..60: note = Description of Artificial Sequence: Syntheticprobe
  source 1..60: mol_type = other DNA
ttagattaagtctggtgccatttttttttttttttagtttctgctttgctgtgtgggggt

SEQ ID NO: 16 - DNA, 60 bp, synthetic construct; identical to SEQ ID NO: 13
  misc_feature 1..60: note = Description of Artificial Sequence: Syntheticprobe
  source 1..60: mol_type = other DNA

SEQ ID NO: 17 - DNA, 24 bp, synthetic construct
  misc_feature 1..24: note = Description of Artificial Sequence: Syntheticprimer
  source 1..24: mol_type = other DNA
cccgtcgctatcaaggaattaaga

SEQ ID NO: 18 - DNA, 24 bp, synthetic construct
  misc_feature 1..24: note = Description of Artificial Sequence: Syntheticprimer
  source 1..24: mol_type = other DNA
caagcagaagacggcatacgagat

SEQ ID NO: 19 - DNA, 20 bp, synthetic construct
  misc_feature 1..20: note = Description of Artificial Sequence: Syntheticprimer
  source 1..20: mol_type = other DNA
aatgatacggcgaccaccga

SEQ ID NO: 20 - DNA, 94 bp, synthetic construct; identical to SEQ ID NO: 11
  misc_feature 1..94: note = Description of Artificial Sequence: Syntheticprobe
  source 1..94: mol_type = other DNA

SEQ ID NO: 21 - DNA, 85 bp, synthetic construct
  misc_feature 1..85: note = Description of Artificial Sequence: Syntheticprobe
  source 1..85: mol_type = other DNA
ttttttggcaccagacttaatctaagcagagaacatgataagagatggcaccagacttaatctaagcagagaacatgataagaga

SEQ ID NO: 22 - DNA, 60 bp, synthetic construct; identical to SEQ ID NO: 12
  misc_feature 1..60: note = Description of Artificial Sequence: Syntheticprobe
  source 1..60: mol_type = other DNA

SEQ ID NO: 23 - DNA, 60 bp, synthetic construct; identical to SEQ ID NO: 13
  misc_feature 1..60: note = Description of Artificial Sequence: Syntheticprobe
  source 1..60: mol_type = other DNA

SEQ ID NO: 24 - DNA, 60 bp, synthetic construct; identical to SEQ ID NO: 14
  misc_feature 1..60: note = Description of Artificial Sequence: Syntheticprobe
  source 1..60: mol_type = other DNA

SEQ ID NO: 25 - DNA, 60 bp, synthetic construct; identical to SEQ ID NO: 15
  misc_feature 1..60: note = Description of Artificial Sequence: Syntheticprobe
  source 1..60: mol_type = other DNA